European Patent Specification EP 3 946 636 B1, published October 15, 2025. Title: CAR for use in the treatment of HvG disease. Applicant: Medizinische Hochschule Hannover Technische Universität Braunschweig. The sequence listing filed with the application follows.

SEQUENCE LISTING (11 sequences)

SEQ ID NO: 1 - protein, 81 aa, Artificial Sequence
  CD8 hinge domain and transmembran domain
FVPVFLPAKPTTTPAPRPPTPAPTIASQPLSLRPEASRPAAGGAVHTRGLDFADIYIWAPLAGTCGVLLLSLVITLYCNHR

SEQ ID NO: 2 - protein, 42 aa, Artificial Sequence
  CD28 signalling domain
WVRSKRSRLLHSDYMNMTPRRPGPTRKHYQPYAPPRDFAAYR

SEQ ID NO: 3 - protein, 113 aa, Artificial Sequence
  CD3zeta signalling domain
RVKFSRSADAPAYQQGQNQLYNELNLGRREEYDVLDKRRGRDPEMGGKPRRKNPQEGLYNELQKDKMAEAYSEIGMKGERRRGKGHDGLYQGLSTATKDTYDALHMQALPPRS

SEQ ID NO: 4 - protein, 280 aa, Artificial Sequence
  hΔFC IgG domain
MGAGATGRAMDGPRLLLLLLLGVSLGGAKEACPTGLYTHSGECCKACNLGEGVAQPCGANQTVCEPCLDSVTFSDVVSATEPCKPCTECVGLQSMSAPCVEADDAVCRCAYGYYQDETTGRCEACRVCEAGSGLVFSCQDKQNTVCEECPDGTYSDEANHVDPCLPCTVCEDTERQLRECTRWADAECEEIPGRWITRSTPPEGSDSTAPSTQEPEAPPEQDLIASTVAGVVTTVMGSSQPVVTRGTTDNLIPVYCSILAAVVVGLVAYIAFKRWNRGIL

SEQ ID NO: 5 - protein, 184 aa, Artificial Sequence
  hCD28 transmembrane domain - hCD3zeta signalling domain
DPKFWVLVVVGGVLACYSLLVTVAFIIFWVRSKRSRLLHSDYMNMTPRRPGPTRKHYQAYAAARDFAAYRSLRVKFSRSADAPAYQQGQNQLYNELNLGRREEYDVLDKRRGRDPEMGGKPRRKNPQEGLYNELQKDKMAEAYSEIGMKGERRRGKGHDGLYQGLSTATKDTYDALHMQALPPR

SEQ ID NO: 6 - protein, 452 aa, Artificial Sequence
  fusion P2A hFOXP3
GATNFSLLKQAGDVEENPGPSMPNPRPGKPSAPSLALGPSPGASPSWRAAPKASDLLGARGPGGTFQGRDLRGGAHASSSSLNPMPPSQLQLPTLPLVMVAPSGARLGPLPHLQALLQDRPHFMHQLSTVDAHARTPVLQVHPLESPAMISLTPPTTATGVFSLKARPGLPPGINVASLEWVSREPALLCTFPNPSAPRKDSTLSAVPQSSYPLLANGVCKWPGCEKVFEEPEDFLKHCQADHLLDEKGRAQCLLQREMVQSLEQQLVLEKEKLSAMQAHLAGKMALTKASSVASSDKGSCCIVAAGSQGPVVPAWSGPREAPDSLFAVRRHLWGSHGNSTFPEFLHNMDYFKFHNMRPPFTYATLIRWAILEAPEKQRTLNEIYHWFTRMFAFFRNHPATWKNAIRHNLSLHKCFVRVESEKGAVWTVDELEFRKKRSQRPSRCSNPTPGP

SEQ ID NO: 7 - protein, 280 aa, Artificial Sequence; identical to SEQ ID NO: 4
  ΔLNGFR (reporter)

SEQ ID NO: 8 - protein, 21 aa, Artificial Sequence
  secretory leader peptide
MALPVTALLLPLALLLHAAAP

SEQ ID NO: 9 - protein, 246 aa, Artificial Sequence
  CHAIN 1..123: heavy chain variable region
  scFv (ELFA*2)
  CHAIN 26..33: CDR1
  CHAIN 51..58: CDR2
  CHAIN 97..112: CDR3
  CHAIN 124..139: linker
  CHAIN 140..246: light chain variable kappa
  CHAIN 166..171: CDR1
  CHAIN 189..191: CDR2
  CHAIN 228..237: CDR3
QVQLVQSGGGVVQPGGSLRVSCAASGVTLSDYGMHWVRQAPGKGLEWVAFIRNDGSDKYYADSVKGRFTISRDNSEKTVSLQMSSLRAEDTAVYYCAKNGESGPLDYWYLDLWGRGTLVTVSSGGGGSGGGGSGGGGSTDVVMTQSPSSLSASVGDRVTITCQSSLDISHYLNWYQQKPGKAPKLLIYDASNLETGVPSRFSGSGSGTHFTFTISSLQPEDFATYYCQQYDNLPLTFGGGTKLEIK

SEQ ID NO: 10 - protein, 21 aa, Artificial Sequence
  CD28 extracellular domain signal peptide
MALPVTALLLPLALLLHAAAP

SEQ ID NO: 11 - protein, 245 aa, Artificial Sequence
  CHAIN 1..123: heavy chain variable region
  variant ELFA*2
  CHAIN 124..138: linker
  CHAIN 139..245: light chain varible kappa
QVQLVQSGGGVVQPGGSLRVSCAASGVTLSDYGMHWVRQAPGKGLEWVAFIRNDGSDKYYADSVKGRFTISRDNSEKTVSLQMSSLRAEDTAVYYCAKNGESGPLDYWYLDLWGRGTLVTVSSGGGGSGGGGSGGGGSDVVMTQSPSSLSASVGDRVTITCQSSLDISHYLNWYQQKPGKAPKLLIYDASNLETGVPSRFSGSGSGTHFTFTISSLQPEDFATYYCQQYDNLPLTFGGGTKLEIK